European Patent Specification EP 4 419 710 B1, published July 2, 2025. Title: PRE-LIBRARY TARGET ENRICHMENT FOR NUCLEIC ACID SEQUENCING. Applicant: IDbyDNA Inc. The sequence listing filed with the application follows.

SEQUENCE LISTING (59 sequences)

SEQ ID NO: 1 - DNA, 582 bp, E. coli
  source 1..582: mol_type = genomic DNA
atgaattttttagctcacctgcatttagcccatctcgcggaaagctcgctttccggcaatttactggctgatttcgtacgcggaaatcctgaagaaagttttccgcccgacgtcgtggctggcattcatatgcatcggcgaatcgacgtattaaccgacaatctgccagaagtccgcgaagcgcgggagtggtttcgtaatgaaacgcgccgtgtcgcgcctattacgctggatgtgatgtgggatcactttctgtcccgccactggtcgcagctgtcgcccgattttccgctacaggaatttacctgttatgcccgggagcaagtgatgactattcttccagactcaccgccacgctttatcaatctgaacaactacttatggtcagagcagtggttggtgcgctatcgcgatatggatttcatccagagcgtgttaaacggcatggcaagccgtcgcccacgtctggatgccctgcgtgactcctggtacgatttagacgcccattacgatgctctcgaaacccgcttctggcagttttatccgcggatgatggagcaggcgtcacgcaaggcgttataa

SEQ ID NO: 2 - DNA, 819 bp, E. coli
  source 1..819: mol_type = genomic DNA
atgcagctaagaattaccagtcgaaaaaaactcaccgctctattatgcgctcttgggctaatttccatcgttgcaatttatccgcgtcagacggtgaattttttctattcgacagcagttcagattacagactacatccacttctacggttatcgcccggttaaatctttcgctattcatattcctgccagttacaccattcacggaatagatgtttcgcgctggcaggagcggatcgactggcagcgggtggcaaaaatgcgcgataacggtatccgcttacaatttgcctttatcaaggcgacggaaggcgaaaagctggtggacccctatttttcgcgtaactggcaactaagccgcgaaaatggcctgctgcgcggggcgtatcattatttctccccgtcggtagcagcgcctgttcaggcgcgattatttctgcaaacggtggatttctcacaaggcgatttccctgccgtgctggacgtagaagaacggggaaaattatcggcaaaagaattacgcaagcgggtaagtcagtggctaaaaatggtcgaaaaaagtacgggaaaaaagccggttatttactcaggagccgttttttatcacaccaatctggcgggctatttcaatgaatatccgtggtgggtggctcactactatcaacgtcgcccggacaatgacggcatggcctggcgtttctggcagcattccgaccgtgggcaggtagatggcattaatggttcggtggattttaatgtgtttaatggcacagaggaggagttgcaggcattcgttgatgggattaaagaaacgccttaa

SEQ ID NO: 3 - DNA, 915 bp, E. coli
  source 1..915: mol_type = genomic DNA
atgagctggattgaacgaattaaaagcaacattactcccacccgcaaggcgagcattcctgaaggggtgtggactaagtgtgatagctgcggtcaggttttataccgcgctgagctggaacgtaatcttgaggtctgtccgaagtgtgaccatcacatgcgtatgacagcgcgtaatcgcctgcatagcctgttagatgaaggaagccttgtggagctgggtagcgagcttgagccgaaagatgtgctgaagtttcgtgactccaagaagtataaagaccgtctggcatctgcgcagaaagaaaccggcgaaaaagatgcgctggtggtgatgaaaggcactctgtatggaatgccggttgtcgctgcggcattcgagttcgcctttatgggcggttccatggggtctgtggtaggtgcgcgtttcgtgcgtgccgttgagcaggcgctggaagataactgcccactgatctgcttctccgcctctggtggcgcacgtatgcaggaagcactgatgtcgctgatgcagatggcgaaaacctctgcggcactggcaaaaatgcaggagcgcggcttgccgtacatctccgtgctgaccgacccgaccatgggcggtgtttctgcaagtttcgccatgctgggcgatctcaacatcgctgaaccgaaagcgttaattggctttgccggtccgcgtgttatcgaacagactgttcgcgaaaaactgccgccaggattccagcgcagtgaattcctgatcgagaaaggcgcgatcgacatgatcgtccgtcgtccggaaatgcgtctgaaactggcgagcattctggcgaagttgatgaatctgccagcgccgaatcctgaagcgccgcgtgaaggcgtagtggtgccaccggtaccggatcaggaacctgaggcctga

SEQ ID NO: 4 - DNA, 40 bp, synthetic construct
  misc_feature 1..40: note = T is 2-sT, W is replacing T or some of the T bases with W-base, and A is 2-amA
  source 1..40: mol_type = other DNA
attacgaaaccactcccgcgcttcgcggacttctggcaga

SEQ ID NO: 5 - DNA, 40 bp, synthetic construct
  source 1..40: mol_type = other DNA
  misc_feature 1..40: note = T is 2-sT, W is replacing T or some of the T bases with W-base, and A is 2-amA
gtttgcagaaataatcgcgcctgaacaggcgctgctaccg

SEQ ID NO: 6 - DNA, 40 bp, synthetic construct
  source 1..40: mol_type = other DNA
  misc_feature 1..40: note = T is 2-sT, W is replacing T or some of the T bases with W-base, and A is 2-amA
ttcctgcatacgtgcgccaccagaggcggagaagcagatc

SEQ ID NO: 7 - DNA, 40 bp, synthetic construct; identical to SEQ ID NO: 4
  source 1..40: mol_type = other DNA
  misc_feature 1..40: note = T is 2-sT, W is replacing T or some of the T bases with W-base, and A is 2-amA

SEQ ID NO: 8 - DNA, 40 bp, synthetic construct; identical to SEQ ID NO: 5
  source 1..40: mol_type = other DNA
  misc_feature 1..40: note = T is 2-sT, W is replacing T or some of the T bases with W-base, and A is 2-amA

SEQ ID NO: 9 - DNA, 40 bp, synthetic construct; identical to SEQ ID NO: 6
  source 1..40: mol_type = other DNA
  misc_feature 1..40: note = T is 2-sT, W is replacing T or some of the T bases with W-base, and A is 2-amA

SEQ ID NO: 10 - DNA, 40 bp, synthetic construct; identical to SEQ ID NO: 4
  source 1..40: mol_type = other DNA
  misc_feature 1..40: note = T is 2-sT, W is replacing T or some of the T bases with W-base, and A is 2-amA

SEQ ID NO: 11 - DNA, 40 bp, synthetic construct; identical to SEQ ID NO: 5
  source 1..40: mol_type = other DNA
  misc_feature 1..40: note = T is 2-sT, W is replacing T or some of the T bases with W-base, and A is 2-amA

SEQ ID NO: 12 - DNA, 40 bp, synthetic construct; identical to SEQ ID NO: 6
  source 1..40: mol_type = other DNA
  misc_feature 1..40: note = T is 2-sT, W is replacing T or some of the T bases with W-base, and A is 2-amA

SEQ ID NO: 13 - DNA, 40 bp, synthetic construct; identical to SEQ ID NO: 4
  source 1..40: mol_type = other DNA
  misc_feature 1..40: note = T is 2-sT, W is replacing T or some of the T bases with W-base, and A is 2-amA

SEQ ID NO: 14 - DNA, 40 bp, synthetic construct; identical to SEQ ID NO: 5
  source 1..40: mol_type = other DNA
  misc_feature 1..40: note = T is 2-sT, W is replacing T or some of the T bases with W-base, and A is 2-amA

SEQ ID NO: 15 - DNA, 40 bp, synthetic construct; identical to SEQ ID NO: 6
  source 1..40: mol_type = other DNA
  misc_feature 1..40: note = T is 2-sT, W is replacing T or some of the T bases with W-base, and A is 2-amA

SEQ ID NO: 16 - DNA, 40 bp, synthetic construct
  source 1..40: mol_type = other DNA
  misc_feature 1..40: note = T is 2-sT, W is replacing T or some of the T bases with W-base, and A is 2-amA
awwacgaaaccacwcccgcgcwwcgcggacwwcwggcaga

SEQ ID NO: 17 - DNA, 40 bp, synthetic construct
  source 1..40: mol_type = other DNA
  misc_feature 1..40: note = T is 2-sT, W is replacing T or some of the T bases with W-base, and A is 2-amA
gwwwgcagaaawaawcgcgccwgaacaggcgcwgcwaccg

SEQ ID NO: 18 - DNA, 40 bp, synthetic construct
  source 1..40: mol_type = other DNA
  misc_feature 1..40: note = T is 2-sT, W is replacing T or some of the T bases with W-base, and A is 2-amA
wwccwgcawacgwgcgccaccagaggcggagaagcagawc

SEQ ID NO: 19 - DNA, 40 bp, synthetic construct; identical to SEQ ID NO: 16
  source 1..40: mol_type = other DNA
  misc_feature 1..40: note = T is 2-sT, W is replacing T or some of the T bases with W-base, and A is 2-amA

SEQ ID NO: 20 - DNA, 40 bp, synthetic construct; identical to SEQ ID NO: 17
  source 1..40: mol_type = other DNA
  misc_feature 1..40: note = T is 2-sT, W is replacing T or some of the T bases with W-base, and A is 2-amA

SEQ ID NO: 21 - DNA, 40 bp, synthetic construct; identical to SEQ ID NO: 18
  source 1..40: mol_type = other DNA
  misc_feature 1..40: note = T is 2-sT, W is replacing T or some of the T bases with W-base, and A is 2-amA

SEQ ID NO: 22 - DNA, 40 bp, synthetic construct; identical to SEQ ID NO: 16
  source 1..40: mol_type = other DNA
  misc_feature 1..40: note = T is 2-sT, W is replacing T or some of the T bases with W-base, and A is 2-amA

SEQ ID NO: 23 - DNA, 40 bp, synthetic construct; identical to SEQ ID NO: 17
  source 1..40: mol_type = other DNA
  misc_feature 1..40: note = T is 2-sT, W is replacing T or some of the T bases with W-base, and A is 2-amA

SEQ ID NO: 24 - DNA, 40 bp, synthetic construct; identical to SEQ ID NO: 18
  source 1..40: mol_type = other DNA
  misc_feature 1..40: note = T is 2-sT, W is replacing T or some of the T bases with W-base, and A is 2-amA

SEQ ID NO: 25 - DNA, 40 bp, synthetic construct
  source 1..40: mol_type = other DNA
  misc_feature 1..40: note = T is 2-sT, W is replacing T or some of the T bases with W-base, and A is 2-amA
atwacgaaaccactcccgcgcwwcgcggacttcwggcaga

SEQ ID NO: 26 - DNA, 40 bp, synthetic construct
  source 1..40: mol_type = other DNA
  misc_feature 1..40: note = T is 2-sT, W is replacing T or some of the T bases with W-base, and A is 2-amA
gtwwgcagaaataatcgcgccwgaacaggcgctgcwaccg

SEQ ID NO: 27 - DNA, 40 bp, synthetic construct
  source 1..40: mol_type = other DNA
  misc_feature 1..40: note = T is 2-sT, W is replacing T or some of the T bases with W-base, and A is 2-amA
twcctgcatacgwgcgccaccagaggcggagaagcagatc

SEQ ID NO: 28 - DNA, 40 bp, synthetic construct
  source 1..40: mol_type = other DNA
  misc_feature 1..40: note = T is 2-sT, W is replacing T or some of the T bases with W-base, and A is 2-amA
tctgccagaagtccgcgaagcgcgggagtggtttcgtaat

SEQ ID NO: 29 - DNA, 40 bp, synthetic construct
  source 1..40: mol_type = other DNA
  misc_feature 1..40: note = T is 2-sT, W is replacing T or some of the T bases with W-base, and A is 2-amA
cggtagcagcgcctgttcaggcgcgattatttctgcaaac

SEQ ID NO: 30 - DNA, 40 bp, synthetic construct
  source 1..40: mol_type = other DNA
  misc_feature 1..40: note = T is 2-sT, W is replacing T or some of the T bases with W-base, and A is 2-amA
gatctgcttctccgcctctggtggcgcacgtatgcaggaa

SEQ ID NO: 31 - DNA, 40 bp, synthetic construct; identical to SEQ ID NO: 28
  source 1..40: mol_type = other DNA
  misc_feature 1..40: note = T is 2-sT, W is replacing T or some of the T bases with W-base, and A is 2-amA

SEQ ID NO: 32 - DNA, 40 bp, synthetic construct; identical to SEQ ID NO: 29
  source 1..40: mol_type = other DNA
  misc_feature 1..40: note = T is 2-sT, W is replacing T or some of the T bases with W-base, and A is 2-amA

SEQ ID NO: 33 - DNA, 40 bp, synthetic construct; identical to SEQ ID NO: 30
  source 1..40: mol_type = other DNA
  misc_feature 1..40: note = T is 2-sT, W is replacing T or some of the T bases with W-base, and A is 2-amA

SEQ ID NO: 34 - DNA, 40 bp, synthetic construct; identical to SEQ ID NO: 28
  source 1..40: mol_type = other DNA
  misc_feature 1..40: note = T is 2-sT, W is replacing T or some of the T bases with W-base, and A is 2-amA

SEQ ID NO: 35 - DNA, 40 bp, synthetic construct; identical to SEQ ID NO: 29
  source 1..40: mol_type = other DNA
  misc_feature 1..40: note = T is 2-sT, W is replacing T or some of the T bases with W-base, and A is 2-amA

SEQ ID NO: 36 - DNA, 40 bp, synthetic construct; identical to SEQ ID NO: 30
  source 1..40: mol_type = other DNA
  misc_feature 1..40: note = T is 2-sT, W is replacing T or some of the T bases with W-base, and A is 2-amA

SEQ ID NO: 37 - DNA, 40 bp, synthetic construct; identical to SEQ ID NO: 28
  source 1..40: mol_type = other DNA
  misc_feature 1..40: note = T is 2-sT, W is replacing T or some of the T bases with W-base, and A is 2-amA

SEQ ID NO: 38 - DNA, 40 bp, synthetic construct; identical to SEQ ID NO: 29
  source 1..40: mol_type = other DNA
  misc_feature 1..40: note = T is 2-sT, W is replacing T or some of the T bases with W-base, and A is 2-amA

SEQ ID NO: 39 - DNA, 40 bp, synthetic construct; identical to SEQ ID NO: 30
  source 1..40: mol_type = other DNA
  misc_feature 1..40: note = T is 2-sT, W is replacing T or some of the T bases with W-base, and A is 2-amA

SEQ ID NO: 40 - DNA, 40 bp, synthetic construct
  source 1..40: mol_type = other DNA
  misc_feature 1..40: note = T is 2-sT, W is replacing T or some of the T bases with W-base, and A is 2-amA
wcwgccagaagwccgcgaagcgcgggagwggwwwcgwaaw

SEQ ID NO: 41 - DNA, 40 bp, synthetic construct
  source 1..40: mol_type = other DNA
  misc_feature 1..40: note = T is 2-sT, W is replacing T or some of the T bases with W-base, and A is 2-amA
cggwagcagcgccwgwwcaggcgcgawwawwwcwgcaaac

SEQ ID NO: 42 - DNA, 40 bp, synthetic construct
  source 1..40: mol_type = other DNA
  misc_feature 1..40: note = T is 2-sT, W is replacing T or some of the T bases with W-base, and A is 2-amA
gawcwgcwwcwccgccwcwggwggcgcacgwawgcaggaa

SEQ ID NO: 43 - DNA, 40 bp, synthetic construct; identical to SEQ ID NO: 40
  source 1..40: mol_type = other DNA
  misc_feature 1..40: note = T is 2-sT, W is replacing T or some of the T bases with W-base, and A is 2-amA

SEQ ID NO: 44 - DNA, 40 bp, synthetic construct; identical to SEQ ID NO: 41
  source 1..40: mol_type = other DNA
  misc_feature 1..40: note = T is 2-sT, W is replacing T or some of the T bases with W-base, and A is 2-amA

SEQ ID NO: 45 - DNA, 40 bp, synthetic construct; identical to SEQ ID NO: 42
  source 1..40: mol_type = other DNA
  misc_feature 1..40: note = T is 2-sT, W is replacing T or some of the T bases with W-base, and A is 2-amA

SEQ ID NO: 46 - DNA, 40 bp, synthetic construct; identical to SEQ ID NO: 40
  source 1..40: mol_type = other DNA
  misc_feature 1..40: note = T is 2-sT, W is replacing T or some of the T bases with W-base, and A is 2-amA

SEQ ID NO: 47 - DNA, 40 bp, synthetic construct; identical to SEQ ID NO: 41
  source 1..40: mol_type = other DNA
  misc_feature 1..40: note = T is 2-sT, W is replacing T or some of the T bases with W-base, and A is 2-amA

SEQ ID NO: 48 - DNA, 40 bp, synthetic construct; identical to SEQ ID NO: 42
  source 1..40: mol_type = other DNA
  misc_feature 1..40: note = T is 2-sT, W is replacing T or some of the T bases with W-base, and A is 2-amA

SEQ ID NO: 49 - DNA, 40 bp, synthetic construct
  source 1..40: mol_type = other DNA
  misc_feature 1..40: note = T is 2-sT, W is replacing T or some of the T bases with W-base, and A is 2-amA
tcwgccagaagwccgcgaagcgcgggagtggtwtcgwaat

SEQ ID NO: 50 - DNA, 40 bp, synthetic construct
  source 1..40: mol_type = other DNA
  misc_feature 1..40: note = T is 2-sT, W is replacing T or some of the T bases with W-base, and A is 2-amA
cggwagcagcgcctgtwcaggcgcgattawwtctgcaaac

SEQ ID NO: 51 - DNA, 40 bp, synthetic construct
  source 1..40: mol_type = other DNA
  misc_feature 1..40: note = T is 2-sT, W is replacing T or some of the T bases with W-base, and A is 2-amA
gawctgctwctccgcctcwggtggcgcacgwatgcaggaa

SEQ ID NO: 52 - DNA, 20 bp, synthetic construct
  source 1..20: mol_type = other DNA
gtaagagaattatgcagtgc

SEQ ID NO: 53 - DNA, 20 bp, synthetic construct
  source 1..20: mol_type = other DNA
  misc_feature 1..20: note = A is 2-Amino-dA-CE Phosphoramidite, and T is dW phosphoramidite
gtaagagaattatgcagtgc

SEQ ID NO: 54 - DNA, 20 bp, synthetic construct
  source 1..20: mol_type = other DNA
  misc_feature 1..20: note = A is 2-Amino-dA-CE Phosphoramidite
gtaagagaattatgcagtgc

SEQ ID NO: 55 - DNA, 20 bp, synthetic construct
  source 1..20: mol_type = other DNA
  misc_feature 1..20: note = T is dW phosphoramidite
gtaagagaattatgcagtgc

SEQ ID NO: 56 - DNA, 20 bp, synthetic construct
  source 1..20: mol_type = other DNA
gcactgcataattctcttac

SEQ ID NO: 57 - DNA, 20 bp, synthetic construct
  source 1..20: mol_type = other DNA
  misc_feature 1..20: note = A is 2-Amino-dA-CE Phosphoramidite, and T is dW phosphoramidite
gcactgcataattctcttac

SEQ ID NO: 58 - DNA, 20 bp, synthetic construct
  source 1..20: mol_type = other DNA
  misc_feature 1..20: note = A is 2-Amino-dA-CE Phosphoramidite
gcactgcataattctcttac

SEQ ID NO: 59 - DNA, 20 bp, synthetic construct
  source 1..20: mol_type = other DNA
  misc_feature 1..20: note = T is dW phosphoramidite
gcactgcataattctcttac